European Patent Application EP 4 512 906 A1, published February 26, 2025. Title: 태그멘테이션을 이용한 벡터 삽입위치 검출 및 클론 정량 방법. Applicant: 서울대학교산학협력단. Application KR. The sequence listing filed with the application follows.

SEQUENCE LISTING (4 sequences)

SEQ ID NO: 1 - DNA, 20 bp, synthetic construct
  source 1..20: mol_type = other DNA
agtagtgtgtgcccgtctgt

SEQ ID NO: 2 - DNA, 20 bp, synthetic construct
  source 1..20: mol_type = other DNA
gtctcgtgggctcggagatg

SEQ ID NO: 3 - DNA, 92 bp, synthetic construct
  source 1..92: mol_type = other DNA
aatgatacggcgaccaccgagatctacacnnnnnnnnnntcgtcggcagcgtcagatgtgtataagagacaggacccttttagtcagtgtgg

SEQ ID NO: 4 - DNA, 49 bp, synthetic construct
  source 1..49: mol_type = other DNA
caagcagaagacggcatacgagatnnnnnnnnnngtctcgtgggctcgg